European Patent Application EP 4 289 439 A2, published December 13, 2023. Title: Leuconostoc citreum WiKim0104. Applicant: Liscure Biosciences. The sequence listing filed with the application follows.

SEQUENCE LISTING (1 sequence)

SEQ ID NO: 1 - DNA, 1430 bp, Leuconostoc citreum
gatgaacgctggcggcgtgcctaatacatgcaagtcgaacgcgcagcgagaggtgcttgcacctttcaagcgagtggcgaacgggtgagtaacacgtggataacctgcctcaaggctggggataacatttggaaacagatgctaataccgaataaaacttagtatcgcatgatatcaagttaaaaggcgctacggcgtcacctagagatggatccgcggtgcattagttagttggtggggtaaaggcttaccaagacgatgatgcatagccgagttgagagactgatcggccacattgggactgagacacggcccaaactcctacgggaggctgcagtagggaatcttccacaatgggcgcaagcctgatggagcaacgccgcgtgtgtgatgaaggctttcgggtcgtaaagcactgttgtatgggaagaaatgctaaaatagggaatgattttagtttgacggtaccataccagaaagggacggctaaatacgtgccagcagccgcggtaatacgtatgtcccgagcgttatccggatttattgggcgtaaagcgagcgcagacggttgattaagtctgatgtgaaagcccggagctcaactccggaatggcattggaaactggttaacttgagtgttgtagaggtaagtggaactccatgtgtagcggtggaatgcgtagatatatggaagaacaccagtggcgaaggcggcttactggacaacaactgacgttgaggctcgaaagtgtgggtagcaaacaggattagataccctggtagtccacaccgtaaacgatgaatactaggtgttaggaggtttccgcctcttagtgccgaagctaacgcattaagtattccgcctggggagtacgaccgcaaggttgaaactcaaaggaattgacggggacccgcacaagcggtggagcatgtggtttaattcgaagcaacgcgaagaaccttaccaggtcttgacatcctttgaagcttttagagatagaagtgttctcttcggagacaaagtgacaggtggtgcatggtcgtcgtcagctcgtgtcgtgagatgttgggttaagtcccgcaacgagcgcaacccttattgttagttgccagcattcagttgggcactctagcgagactgccggtgacaaaccggaggaaggcggggacgacgtcagatcatcatgccccttatgacctgggctacacacgtgctacaatggcgtatacaacgagttgccaacctgcgaaggtgagctaatctcttaaagtacgtctcagttcggactgcagtctgcaactcgactgcacgaagtcggaatcgctagtaatcgcggatcagcacgccgcggtgaatacgttcccgggtcttgtacacaccgcccgtcacaccatgggagtttgtaatgcccaaagccggtggcctaacc